European Patent Application EP 4 635 967 A1, published October 22, 2025. Title: 包含亲脂性单体的寡核苷酸以及其在非肝递送中的应用. Applicant: 上海拓界生物医药科技有限公司. Application WO, filed December 13, 2023. The sequence listing filed with the application follows.

SEQUENCE LISTING (66 sequences)

SEQ ID NO: 1 - RNA, 21 nt, synthetic construct
  source 1..21: mol_type = other RNA
gtgctttaactacaatataca

SEQ ID NO: 2 - RNA, 23 nt, synthetic construct
  source 1..23: mol_type = other RNA
tgtatattgtagttaaagcacat

SEQ ID NO: 3 - RNA, 21 nt, synthetic construct
  source 1..21: mol_type = other RNA
  modified_base 1..21: mod_base = OTHER; note = with modifications as shown in Table 2 TJR10072 SS chain; note (original language) = 具有如表2 TJR10072 SS链所示的修饰
gtgctttaactacaatataca

SEQ ID NO: 4 - RNA, 23 nt, synthetic construct
  source 1..23: mol_type = other RNA
  modified_base 1..23: mod_base = OTHER; note = with modifications as shown in Table 2 TJR10072 AS chain; note (original language) = 具有如表2 TJR10072 AS链所示的修饰
tgtatattgtagttaaagcacat

SEQ ID NO: 5 - RNA, 21 nt, synthetic construct
  source 1..21: mol_type = other RNA
  modified_base 1..21: mod_base = OTHER; note = with modifications as shown in Table 2 TJR10073 SS chain; note (original language) = 具有如表2中TJR10073 SS链所示的修饰
gtgctttaactacaatataca

SEQ ID NO: 6 - RNA, 23 nt, synthetic construct
  source 1..23: mol_type = other RNA
  modified_base 1..23: mod_base = OTHER; note = with the sequence shown in Table 2 TJR100073 AS chain; note (original language) = 具有如表2 中TJR100073 AS链所示的序列
tgtatattgtagttaaagcacat

SEQ ID NO: 7 - RNA, 21 nt, synthetic construct
  source 1..21: mol_type = other RNA
  modified_base 1..21: mod_base = OTHER; note = with the sequence shown in Table 2 TJR100344 SS chain; note (original language) = 具有如表2中TJR100344 SS链所示的序列
gtgctttaactacaatataca

SEQ ID NO: 8 - RNA, 23 nt, synthetic construct
  source 1..23: mol_type = other RNA
  modified_base 1..23: mod_base = OTHER; note = with the sequence shown in Table 2 TJR100344 AS chain; note (original language) = 具有如表2中TJR100344 AS链所示的序列
tgtatattgtagttaaagcacat

SEQ ID NO: 9 - RNA, 21 nt, synthetic construct
  source 1..21: mol_type = other RNA
  modified_base 1..21: mod_base = OTHER; note = with the modifications shown in Table 2 TJR100345 SS chain; note (original language) = 具有如表2中TJR100345 SS链所示的修饰
gtgctttaactacaatataca

SEQ ID NO: 10 - RNA, 23 nt, synthetic construct
  source 1..23: mol_type = other RNA
  modified_base 1..23: mod_base = OTHER; note = with the modifications shown in Table 2 TJR100345 AS chain; note (original language) = 具有如表2中TJR100345 AS链所示的修饰
tgtatattgtagttaaagcacat

SEQ ID NO: 11 - RNA, 21 nt, synthetic construct
  source 1..21: mol_type = other RNA
ccggtcccaggttatgacact

SEQ ID NO: 12 - RNA, 23 nt, synthetic construct
  source 1..23: mol_type = other RNA
agtgtcataacctgggaccggat

SEQ ID NO: 13 - RNA, 21 nt, synthetic construct
  source 1..21: mol_type = other RNA
tcggtcccaggttatgacact

SEQ ID NO: 14 - RNA, 23 nt, synthetic construct
  source 1..23: mol_type = other RNA
agtgtcataacctgggaccgaat

SEQ ID NO: 15 - RNA, 21 nt, synthetic construct
  source 1..21: mol_type = other RNA
  modified_base 1..21: mod_base = OTHER; note = with the modifications shown in Table 4 TJR102160 SS chain; note (original language) = 具有如表4中TJR102160 SS链所示的修饰
ccggtcccaggttatgacact

SEQ ID NO: 16 - RNA, 23 nt, synthetic construct
  source 1..23: mol_type = other RNA
  modified_base 1..23: mod_base = OTHER; note = with the sequence shown in Table 4 TJR102160 AS chain; note (original language) = 具有如表4中TJR102160 AS链所示的序列
agtgtcataacctgggaccggat

SEQ ID NO: 17 - RNA, 21 nt, synthetic construct
  source 1..21: mol_type = other RNA
  modified_base 1..21: mod_base = OTHER; note = with the modifications shown in Table 4 TJR102161; note (original language) = 具有如表4中TJR102161所示的修饰
ccggtcccaggttatgacact

SEQ ID NO: 18 - RNA, 23 nt, synthetic construct
  source 1..23: mol_type = other RNA
  modified_base 1..23: mod_base = OTHER; note = with the modifications shown in Table 4 TJR102161 AS chain; note (original language) = 具有如表4中TJR102161 AS链所示的修饰
agtgtcataacctgggaccggat

SEQ ID NO: 19 - RNA, 21 nt, synthetic construct
  source 1..21: mol_type = other RNA
  modified_base 1..21: mod_base = OTHER; note = with the modifications shown in Table 4 TJR102162 SS chain; note (original language) = 具有如表4中TJR102162 SS链所示的修饰
ccggtcccaggttatgacact

SEQ ID NO: 20 - RNA, 23 nt, synthetic construct
  source 1..23: mol_type = other RNA
  modified_base 1..23: mod_base = OTHER; note = with the modifications shown in Table 4 TJR102162 AS chain; note (original language) = 具有表4中TJR102162 AS链所示的修饰
agtgtcataacctgggaccggat

SEQ ID NO: 21 - RNA, 21 nt, synthetic construct
  source 1..21: mol_type = other RNA
  modified_base 1..21: mod_base = OTHER; note = with the modifications shown in Table 4 TJR102178; note (original language) = 具有如表4中TJR102178所示的修饰
tcggtcccaggttatgacact

SEQ ID NO: 22 - RNA, 23 nt, synthetic construct
  source 1..23: mol_type = other RNA
  modified_base 1..23: mod_base = OTHER; note = with the modifications shown in Table 4 TJR102178 AS chain; note (original language) = 具有如表4中TJR102178 AS链所示的修饰
agtgtcataacctgggaccgaat

SEQ ID NO: 23 - RNA, 21 nt, synthetic construct
  source 1..21: mol_type = other RNA
  modified_base 1..21: mod_base = OTHER; note = with the modifications shown in Table 4 TJR102179 SS chain; note (original language) = 具有如表4中TJR102179 SS链所示的修饰
tcggtcccaggttatgacact

SEQ ID NO: 24 - RNA, 23 nt, synthetic construct
  source 1..23: mol_type = other RNA
  modified_base 1..23: mod_base = OTHER; note = with the modifications shown in Table 4 TJR102179; note (original language) = 具有如表4中TJR102179所示的修饰
agtgtcataacctgggaccgaat

SEQ ID NO: 25 - RNA, 21 nt, synthetic construct
  source 1..21: mol_type = other RNA
  modified_base 1..21: mod_base = OTHER; note = with the modifications shown in Table 4 TJR102180 SS chain; note (original language) = 具有如表4中TJR102180 SS链所示的修饰
tcggtcccaggttatgacact

SEQ ID NO: 26 - RNA, 23 nt, synthetic construct
  source 1..23: mol_type = other RNA
  modified_base 1..23: mod_base = OTHER; note = with the modifications shown in Table 4 TJR102180; note (original language) = 具有表4中TJR102180所示的修饰
agtgtcataacctgggaccgaat

SEQ ID NO: 27 - RNA, 21 nt, synthetic construct
  source 1..21: mol_type = other RNA
cctcctgttgctgagtatcaa

SEQ ID NO: 28 - RNA, 23 nt, synthetic construct
  source 1..23: mol_type = other RNA
ttgatactcagcaacaggaggag

SEQ ID NO: 29 - RNA, 21 nt, synthetic construct
  source 1..21: mol_type = other RNA
  modified_base 1..21: mod_base = OTHER; note = with the modifications shown in Table 6 TJR102149 SS chain; note (original language) = 具有如表6中TJR102149 SS链所示的修饰
cctcctgttgctgagtatcaa

SEQ ID NO: 30 - RNA, 23 nt, synthetic construct
  source 1..23: mol_type = other RNA
  modified_base 1..23: mod_base = OTHER; note = with the modifications shown in Table 6 TJR102149 AS chain; note (original language) = 具有如表6中TJR102149 AS链所示的修饰
ttgatactcagcaacaggaggag

SEQ ID NO: 31 - RNA, 21 nt, synthetic construct
  source 1..21: mol_type = other RNA
  modified_base 1..21: mod_base = OTHER; note = with the modifications shown in Table 6 TJR102150 SS chain; note (original language) = 具有如表6中TJR102150 SS链所示的修饰
cctcctgttgctgagtatcaa

SEQ ID NO: 32 - RNA, 23 nt, synthetic construct
  source 1..23: mol_type = other RNA
  modified_base 1..23: mod_base = OTHER; note = with the modifications shown in Table 6 TJR102150 AS chain; note (original language) = 具有如表6中TJR102150 AS链所示的修饰
ttgatactcagcaacaggaggag

SEQ ID NO: 33 - RNA, 21 nt, synthetic construct
  source 1..21: mol_type = other RNA
  modified_base 1..21: mod_base = OTHER; note = with the modifications shown in Table 6 TJR102151 SS chain; note (original language) = 具有如表6中TJR102151 SS链所示的修饰
cctcctgttgctgagtatcaa

SEQ ID NO: 34 - RNA, 23 nt, synthetic construct
  source 1..23: mol_type = other RNA
  modified_base 1..23: mod_base = OTHER; note = with the modifications shown in Table 6 TJR102151 AS chain; note (original language) = 具有如表6中TJR102151 AS链所示的修饰
ttgatactcagcaacaggaggag

SEQ ID NO: 35 - RNA, 21 nt, synthetic construct
  source 1..21: mol_type = other RNA
ttcactttatcaatagttcca

SEQ ID NO: 36 - RNA, 23 nt, synthetic construct
  source 1..23: mol_type = other RNA
tggaactattgataaagtgaatt

SEQ ID NO: 37 - RNA, 21 nt, synthetic construct
  source 1..21: mol_type = other RNA
ttcactttatcaatagttcct

SEQ ID NO: 38 - RNA, 23 nt, synthetic construct
  source 1..23: mol_type = other RNA
aggaactattgataaagtgaatt

SEQ ID NO: 39 - RNA, 21 nt, synthetic construct
  source 1..21: mol_type = other RNA
  modified_base 1..21: mod_base = OTHER; note = with the modifications shown in Table 8 TJR102217 SS chain; note (original language) = 具有如表8中TJR102217 SS链所示的修饰
ttcactttatcaatagttcca

SEQ ID NO: 40 - RNA, 23 nt, synthetic construct
  source 1..23: mol_type = other RNA
  modified_base 1..23: mod_base = OTHER; note = with the modifications shown in Table 8 TJR102217 AS chain; note (original language) = 具有如表8中TJR102217 AS链所示的修饰
tggaactattgataaagtgaatt

SEQ ID NO: 41 - RNA, 21 nt, synthetic construct
  source 1..21: mol_type = other RNA
  modified_base 1..21: mod_base = OTHER; note = with the modifications shown in Table 8 TJR102218 SS chain; note (original language) = 具有如表8中TJR102218 SS链所示的修饰
ttcactttatcaatagttcca

SEQ ID NO: 42 - RNA, 23 nt, synthetic construct
  source 1..23: mol_type = other RNA
  modified_base 1..23: mod_base = OTHER; note = with the modifications shown in Table 8 TJR102218 AS chain; note (original language) = 具有如表8中TJR102218 AS链所示的修饰
tggaactattgataaagtgaatt

SEQ ID NO: 43 - RNA, 21 nt, synthetic construct
  source 1..21: mol_type = other RNA
  modified_base 1..21: mod_base = OTHER; note = with the modifications shown in Table 8 TJR102219 SS chain; note (original language) = 具有如表8中TJR102219 SS链所示的修饰
ttcactttatcaatagttcca

SEQ ID NO: 44 - RNA, 23 nt, synthetic construct
  source 1..23: mol_type = other RNA
  modified_base 1..23: mod_base = OTHER; note = with the modifications shown in Table 8 TJR102219 AS chain; note (original language) = 具有如表8中TJR102219 AS链所示的修饰
tggaactattgataaagtgaatt

SEQ ID NO: 45 - RNA, 21 nt, synthetic construct
  source 1..21: mol_type = other RNA
  modified_base 1..21: mod_base = OTHER; note = with the modifications shown in Table 8 TJR101646 SS chain; note (original language) = 具有如表8中TJR101646 SS链所示的修饰
ttcactttatcaatagttcca

SEQ ID NO: 46 - RNA, 23 nt, synthetic construct
  source 1..23: mol_type = other RNA
  modified_base 1..23: mod_base = OTHER; note = with the modifications shown in Table 8 TJR101646 AS chain; note (original language) = 具有如表8中TJR101646 AS链所示的修饰
tggaactattgataaagtgaatt

SEQ ID NO: 47 - RNA, 21 nt, synthetic construct
  source 1..21: mol_type = other RNA
  modified_base 1..21: mod_base = OTHER; note = with the modifications shown in Table 8 TJR101647; note (original language) = 具有如表8中TJR101647所示的修饰
ttcactttatcaatagttcca

SEQ ID NO: 48 - RNA, 23 nt, synthetic construct
  source 1..23: mol_type = other RNA
  modified_base 1..23: mod_base = OTHER; note = with the modifications shown in Table 8 TJR101647 AS chain; note (original language) = 具有如表8中TJR101647 AS链所示的修饰
tggaactattgataaagtgaatt

SEQ ID NO: 49 - RNA, 21 nt, synthetic construct
  source 1..21: mol_type = other RNA
  modified_base 1..21: mod_base = OTHER; note = with the modifications shown in Table 8 TJR101740 SS chain; note (original language) = 具有如表8中TJR101740 SS链所示的修饰
ttcactttatcaatagttcca

SEQ ID NO: 50 - RNA, 23 nt, synthetic construct
  source 1..23: mol_type = other RNA
  modified_base 1..23: mod_base = OTHER; note = with the modifications shown in Table 8 TJR101740 SS chain; note (original language) = 具有如表8中TJR101740 SS链所示的修饰
tggaactattgataaagtgaatt

SEQ ID NO: 51 - DNA, 21 bp, synthetic construct
  source 1..21: mol_type = other DNA
aggtcggtgtgaacggatttg

SEQ ID NO: 52 - DNA, 19 bp, synthetic construct
  source 1..19: mol_type = other DNA
ggggtcgttgatggcaaca

SEQ ID NO: 53 - DNA, 20 bp, synthetic construct
  source 1..20: mol_type = other DNA
tccctagcatgagcgcctta

SEQ ID NO: 54 - DNA, 20 bp, synthetic construct
  source 1..20: mol_type = other DNA
ccacgacgcagttggatgtt

SEQ ID NO: 55 - DNA, 20 bp, synthetic construct
  source 1..20: mol_type = other DNA
gacagacagcacaccctaaa

SEQ ID NO: 56 - DNA, 20 bp, synthetic construct
  source 1..20: mol_type = other DNA
cacacggaggtgtgtcataa

SEQ ID NO: 57 - DNA, 24 bp, synthetic construct
  source 1..24: mol_type = other DNA
atcccaagaaagccgctcagatcc

SEQ ID NO: 58 - DNA, 24 bp, synthetic construct
  source 1..24: mol_type = other DNA
gaccccttcattgacctcaactac

SEQ ID NO: 59 - DNA, 20 bp, synthetic construct
  source 1..20: mol_type = other DNA
ttgacggtgccatggaattt

SEQ ID NO: 60 - DNA, 22 bp, synthetic construct
  source 1..22: mol_type = other DNA
ttacatgttccaatatgattcc

SEQ ID NO: 61 - DNA, 22 bp, synthetic construct
  source 1..22: mol_type = other DNA
gtggcatctcaactcggattac

SEQ ID NO: 62 - DNA, 22 bp, synthetic construct
  source 1..22: mol_type = other DNA
cgtttccgcaagatcacataga

SEQ ID NO: 63 - DNA, 24 bp, synthetic construct
  source 1..24: mol_type = other DNA
ctacggtttcgcctacatcctggc

SEQ ID NO: 64 - DNA, 23 bp, synthetic construct
  source 1..23: mol_type = other DNA
ctctcaggtttgtggaggtaatc

SEQ ID NO: 65 - DNA, 23 bp, synthetic construct
  source 1..23: mol_type = other DNA
ccagggttcttaggaggtatttg

SEQ ID NO: 66 - DNA, 14 bp, synthetic construct
  source 1..14: mol_type = other DNA
cttctcttcctgct